European Patent Application EP 4 303 325 A1, published January 10, 2024. Title: A METHOD FOR DETERMINING BACTERIAL METABOLITES FOR INDIVIDUALIZED NUTRITIONAL ADJUSTMENT. Applicant: Max-Delbrück-Centrum für Molekulare Medizin in der Helmholtz-Gemeinschaft. The sequence listing filed with the application follows.

SEQUENCE LISTING (100 sequences)

SEQ ID NO: 1 - DNA, 113 bp, Eubacterium rectale
  source 1..113: mol_type = genomic DNA
  primer_bind 6..23
  primer_bind 91..107
ttattcggtggatacggatatatccgtgagtatgatgtagagcgtatgatgcgtgatgctaagattacagagatctacgagggaacttcagaggttcagcgtatggttatttc

SEQ ID NO: 2 - DNA, 190 bp, Faecalibacterium prausnitzii
  source 1..190: mol_type = genomic DNA
  primer_bind 73..90
  primer_bind 149..166
acaggctaagctgatcgcagcccgcactgcaagcgatgtgacccgccgctgcctgcagctgttcggtggttacggctacacccgtgactaccccatcgagcgcatgatgcgtgatgccaagatcactgagatctacgagggcaccagcgaagtgcagatgatggtcatttccggcgcgctgctgaagtaa

SEQ ID NO: 3 - DNA, 114 bp, Anaerobutyricum hallii
  source 1..114: mol_type = genomic DNA
  primer_bind 7..22
  primer_bind 90..108
ttatatggtggatatggatatacaaaagattatccaatcgagagaatgatgcgtgacgctaagattacagaaatctatgaaggaacttctgaagtacagatgatggttatctct

SEQ ID NO: 4 - DNA, 114 bp, Roseburia faecis
  source 1..114: mol_type = genomic DNA
  primer_bind 7..22
  primer_bind 91..108
ttattcggtggatacggatatatccgtgagtacgacgtagagcgtatgatgcgcgatgccaagatcacagagatctacgaaggaacttccgaagttcagcgtatggttatttct

SEQ ID NO: 5 - DNA, 114 bp, Roseburia inulinivorans
  source 1..114: mol_type = genomic DNA
  primer_bind 7..23
  primer_bind 91..108
ttattcggtggatatggatacatcagagagtacgatgtagagcgtatgatgcgtgatgctaagatcacagagatctatgagggaacaagcgaagtacagcgcatggttatctca

SEQ ID NO: 6 - DNA, 114 bp, Coprococcus eutactus
  source 1..114: mol_type = genomic DNA
  primer_bind 7..23
  primer_bind 91..108
ttacacggtggttacggttacatcaaggagtacgatgttgagcgtatgatgcgtgatgctaagattacagagatctacgagggaacttcagaggttcagcgtatggttatttct

SEQ ID NO: 7 - DNA, 113 bp, Oscillibacter sp.
  source 1..113: mol_type = genomic DNA
  primer_bind 7..23
  primer_bind 91..107
ctattcggcggctatggctacacccgtgaatatcccgtggagcggatgatgcgagacgccaagatcactgagatctacgagggtaccagcgaggtccagcgcatggtgatctc

SEQ ID NO: 8 - DNA, 17 bp, synthetic construct
  source 1..17: mol_type = other DNA; note = Primer
ggygghtaygghtayay

SEQ ID NO: 9 - DNA, 18 bp, synthetic construct
  source 1..18: mol_type = other DNA; note = Primer
tggatctcaagagaatat

SEQ ID NO: 10 - DNA, 18 bp, synthetic construct
  source 1..18: mol_type = other DNA; note = Primer
cggctacacccgtgacta

SEQ ID NO: 11 - DNA, 17 bp, synthetic construct
  source 1..17: mol_type = other DNA; note = Primer
accatvmkstgnacytc

SEQ ID NO: 12 - DNA, 17 bp, synthetic construct
  source 1..17: mol_type = other DNA; note = Primer
atagcttcggatgtacc

SEQ ID NO: 13 - DNA, 21 bp, synthetic construct
  source 1..21: mol_type = other DNA; note = Primer
accggaaatgaccatcatctg

SEQ ID NO: 14 - DNA, 24 bp, synthetic construct
  source 1..24: mol_type = other DNA; note = Probe
tgatgcghgaygcyaagatyacwg

SEQ ID NO: 15 - DNA, 22 bp, synthetic construct
  source 1..22: mol_type = other DNA; note = Probe
tgtatcgtgatgcaaagatcac

SEQ ID NO: 16 - DNA, 20 bp, synthetic construct
  source 1..20: mol_type = other DNA; note = Probe
atgatgcgygatgcyaagat

SEQ ID NO: 17 - DNA, 464 bp, Bacteroides vulgatus
  source 1..464: mol_type = genomic DNA
  primer_bind 7..26
  primer_bind 431..458
acgaactggctcacaaggcttgggaacatattcaggaaattgaaagcttgggcggtatggcaaaagctatcgaaaccggagtacccaaaatgcgtattgaagaagctgcggcacgtactcaggcccgtatcgactccggtgcccagacaattgtcggcactaacaaatatcgtttggaaaaagaggatcctatcgatatccttgaagtagacaatacagccgtacgtttggaacaaattgaaaatctgaagcgtttgaaagaaggccgcaatcaagcagaagtagacaaagctttggcagccatcaccgaatgtgtaaagacaggtaaaggcaatttgctggaactggctgtagaggcagctcatgtccgtgctaccttgggcgagatttcggatgcttgtgaaacaattgtaggacgttataaagcagtaatcagaactatatcaggcgtgtactcatcagaa

SEQ ID NO: 18 - DNA, 464 bp, Bacteroides acidifaciens
  source 1..464: mol_type = genomic DNA
  primer_bind 7..26
  primer_bind 431..458
acgaactggctcataaggcttgggaacacattcaggaaatcgaaaaactgggcggtatggcgaaagctatcgaaaccggaattccgaaaatgcgtatcgaagaagctgccgcacgtacacaggctcgtatcgacagtggtcagcagactattgtgggtgtgaacaagtatcgtctggataaagaagctccgattgatattcttgaaattgataatactgccgttcgtcttgaacagattgaaaacctgaaacgtttgaaagaaggacgcaaccaggctgaagtggacaaggcattggctgcaattaccgaatgtgtgaaaaccggtaagggcaacttgctggaactggctgtggaagcggctcgtgttcgtgcgacattgggtgaaatctcatctgcttgcgaacagattgtaggacgttataaagcaataattagaactatatcaggcgtgtattcatcagaa

SEQ ID NO: 19 - DNA, 464 bp, Bacteroides thetaiotaomicron
  source 1..464: mol_type = genomic DNA
  primer_bind 7..26
  primer_bind 431..458
acgaactggctcacaaggcttgggaacgtatcgaggaagtagaaaaactgggtggtatggcgaaagctatcgagaccggtattcctaagatgcgtatcgaagaggctgctgctcgtacgcaggcccgtatcgacagcggttctcagactattgttggtgtgaacaaatatcgtctggaaaaagaagctccgattgatatccttgagattgataacacggcagttcgtcttgaacagatcgagaacctgaaacgtttgaaagaaggacgtaaccaggcagaagtggacaaagcactggcagccatcaccgaatgcgtggagaccggtaagggtaacttgctggaactggctgtagaagctgctcgtgttcgtgcaacgctgggtgaaatctcctatgcttgcgaaaaggttgtaggacgttataaagcaataattagaacaatatcaggcgtgtattcatcagaa

SEQ ID NO: 20 - DNA, 464 bp, Bacteroides ovatus
  source 1..464: mol_type = genomic DNA
  primer_bind 7..26
  primer_bind 431..458
acgaactggcacacaaggcttgggagcatattcaggaaattgaaaaactgggtggtatggcgaaagctatcgaaacaggtattccaaagatgcgtatcgaagaagctgctgcccgtacacaggctcgtatcgacagtggtcagcaaacaattgtgggtgtgaacaagtatcgtttggaaaaagaagctccgattgatattcttgaaattgataatactgcagtccgtcttgaacagatcgaaaacctgaaacgtttgaaagaaggacgtaatcaggctgaagtggacaaagcattggcagctatcactgaatgtgtgaagaccggcaagggtaacttgcttgaactggcagttgaagcagctcgtgttcgcgcaacattgggtgagatttcttatgcttgcgaacagatagtaggacgttataaagcaataattagaacgatatcaggcgtgtattcatcagaa

SEQ ID NO: 21 - DNA, 464 bp, Bacteroides intestinalis
  source 1..464: mol_type = genomic DNA
  primer_bind 7..26
  primer_bind 431..458
atgacttggctcacaaggcttgggagcttattcaggaagtagaaaaactgggtggtatggcaaaggctatcgaaaccggtattcctaagatgcgcatcgaagaagctgctgcacgtacacaggctcgtatcgactccggttctcagactattgttggtgtgaataaatatcgtctggagaaagaagctccgattgatatcctcgaaatcgacaatacggctgttcgtctggaacagattgagaacctgaagcgcttgaaagaaggaagaaatgaggctgaagtgcagaaagcattggaagctattaccaaatgcgtggaaaccaaggaaggcaatttgctggagctggcagtagaagctgcccgtgttcgcgctacgttgggagaaatctcttatgcttgcgaaaagattgtaggacgttataaggcaataatcagaactatatcaggcgtgtattcatcagaa

SEQ ID NO: 22 - DNA, 464 bp, Bacteroides uniformis
  source 1..464: mol_type = genomic DNA
  primer_bind 7..26
  primer_bind 431..458
atgagttggctcacaaggcttgggagttgattcaggaagtagagaaactgggcggtatggcaaaagccatcgaaaccggcattcccaaaatgcgtatcgaagaggctgctgcgcgtacacaagcccgtatcgacagcggttcacagaccattgtcggtgtgaacaagtatcgtctggagaaagaagctccgattgatattcttgaaattgacaatacggcagtccgtcaggaacagattgagaacctgaagcgtctgaaggaaggacgtaaccaggcggaagtggacaaggcattggaggctattactgaatgtgtaaagaccggtaagggaaacttgctggaactggcagtcgaggcagcccgtgtccgtgccactttgggggaaatctcttatgcttgcgaaaagattgtaggacgttataaagcagtaattagaactatatcaggcgtgtattcatcagaa

SEQ ID NO: 23 - DNA, 465 bp, Bacteroides fragilis
  source 1..465: mol_type = genomic DNA
  primer_bind 8..27
  primer_bind 432..459
aatgaattggctcacagtgcttgggagcatattcaggaaatcgagaagttgggaggtatggcaaaggctatcgagaccggtattccgaaaatgcgtatcgaagaagcggctgcccgtgcacaagcacgtatcgacagcggatcgcagaccattgtcggtgtaaataagtatcgtcttgaaaaagaagatccgattgatattcttgaagtagacaatactgctgttcgtaaagagcagatcgagaacctgaaacgtttgaaagaaggtcgtaatcaggccgaagtggacaaggcactggccgctatcactgaatgtgtgaaaaccggtaagggcaatttgctcgagttggcggtagaagctgcccgtgttcgtgctacattgggtgaaatctcgtatgcttgcgaacaaatagtaggacgttataaagcaataatcagaactatatcaggcgtgtattcatcagaa

SEQ ID NO: 24 - DNA, 20 bp, synthetic construct
  source 1..20: mol_type = other DNA; note = Primer
tggcwcayarkgcttgggar

SEQ ID NO: 25 - DNA, 28 bp, synthetic construct
  source 1..28: mol_type = other DNA; note = Primer
tgartacacgcctgatathgttctratt

SEQ ID NO: 26 - DNA, 135 bp, Akkermansia muciniphila
  source 1..135: mol_type = genomic DNA
  primer_bind 7..27
  primer_bind 109..129
ggccgtggactccatcctggacatggaaatcctcttcaagggcattcccctggacaaaatgtccgtttccatgaccatgaacggcgccgtgctgcccgtgctggctttctacatcgtcgccgcccaggaacaggg

SEQ ID NO: 27 - DNA, 135 bp, Escherichia coli
  source 1..135: mol_type = genomic DNA
  primer_bind 7..27
  primer_bind 109..129
cgctatcgacaccgtggaagatatgaaagtcctgttcgaccagatcccgctggataaaatgtcggtttcgatgaccatgaatggcgcagtgctaccagtactggcgttttatatcgtcgccgcagaagagcaagg

SEQ ID NO: 28 - DNA, 135 bp, Veillonella parvula
  source 1..135: mol_type = genomic DNA
  primer_bind 7..27
  primer_bind 109..129
tgcagtagactccatcctcgacatggaaattctattctccggtatccctcttgatcaaatgtccgtatccatgacaatgaacggcgccgtattgccagtaatggcgttctacatcttggctggtgaagaacaagg

SEQ ID NO: 29 - DNA, 21 bp, synthetic construct
  source 1..21: mol_type = other DNA; note = Primer
vgacwccrtsswvgayatgga

SEQ ID NO: 30 - DNA, 21 bp, synthetic construct
  source 1..21: mol_type = other DNA; note = Primer
tcytsdscrgcgamgatrtar

SEQ ID NO: 31 - DNA, 37 bp, synthetic construct
  source 1..37: mol_type = other DNA; note = Probe
gaagargckgctgcncgtgcacargchcgtatcgacw

SEQ ID NO: 32 - DNA, 326 bp, Desulfovibrio desulfuricans
  source 1..326: mol_type = genomic DNA
  primer_bind 7..26
  primer_bind 303..322
aagttctttgccggataccagcccttcgtgaacatgtgcgtgggcggcgttacccgtgaaggacgcgacgccaccaacgagctgacctacctgctcatggacgcagtgcgccacgtgcgtatttaccagccctcgctggcaacccgcgtgcacaattcctcgccgcaggaatacctcaagaaaatcgtggccgtcatccgttccggcatgggcttccccgccgtgcactttgacgacacccacatcaagatgatgctggccaagggcgtgagcattgaagacgcccgcgactactgcctcatgggttgcgtggaaccgcagaaagc

SEQ ID NO: 33 - DNA, 20 bp, synthetic construct
  modified_base 6: mod_base = i
  modified_base 9: mod_base = i
  source 1..20: mol_type = other DNA; note = Primer
ttygcnggntaycarccntt

SEQ ID NO: 34 - DNA, 20 bp, synthetic construct
  modified_base 9: mod_base = i
  modified_base 15: mod_base = i
  source 1..20: mol_type = other DNA; note = Primer
tgnggytcnacrcancccat

SEQ ID NO: 35 - DNA, 1149 bp, Desulfovibrio desulfuricans
  source 1..1149: mol_type = genomic DNA
  primer_bind 7..26
  primer_bind 69..88
  primer_bind 130..148
  primer_bind 598..624
  primer_bind 787..805
  primer_bind 1122..1142
ctgtgcactttgacgacacccacatcaagatgatgctggccaagggcgtcgacattgaagacgcccgcgactactgcctcatgggttgcgtggaaccgcaaaaatccggccgcctgtatcagtggacgtccacggcatacacccagtggcccatctgcatcgagcttgtactcaaccgcggcgtgcccctctggtacggcaagcaggtctgccctgacctcggcgatctgagccagttcgacacttttgaaaagtttgatgccgccgtcaaggaacagatcaggtacatcaccaaatggtcaagcgtggctacggttatctcccagcgtgtccaccgcgacctggcgcccaagccgctgatgtccatcatgtacgaaggctgcatggaaaaaggccgcgatgtagccgccggcggtgccatgtacaacttcggtcccggcgtgatctggagcggccttgcaacctacgccgactcgatggccgctatcaagaagctcgtgtatgacgacaggaagtacaccctgcagcaacttaacgaggcgctcaaagccaactttgaaggctatgacgccattctggccgactgcctggccgcgcccaaatacggcaacgatgatgactatgccgacgatatcgccgccgacctcatcgcctttaccgagcgtgagcaccgcaagtaccggacgctctactccatcctgagccacggtacactgtccatttccaacaacacgccctttggtcagctcctgggcgcttcggccggcggccgcaaggcatggcagccgctttccgacggtatcagccccacgcagggcgcggactacaagggtcccacggccatcatcaagagcgtgtccaagatgtccaacgacaacatgaacatcggcatggtgcataacttcaagctcatgcccggcctgctggatacccccgaaggcgaacagggcattatcaccctcattcgctctgccagcatacttggcaacggtgaaatgcagttcaactatctggacaacaagaccatgcttgaagcccagcagaaccccaaagactatcgcgaccttgtggtccgtgtggcaggctatagcgccttctttgtggaactttgcaaggacgtgcaggacgaaatcatcagcagaactgtgc

SEQ ID NO: 36 - DNA, 1148 bp, Klebsiella variicola
  source 1..1148: mol_type = genomic DNA
  primer_bind 7..26
  primer_bind 69..88
  primer_bind 131..148
  primer_bind 598..624
  primer_bind 787..805
  primer_bind 1122..1142
cctgccacttcgatgactcccacatcaagatgatgctgcgcaaaggcttcgattttgaagacgcccgcgattactgcctgatgggctgcgttgagccgcagaaatccgggcgcatctaccagtggacctccaccggctacacccagtggcctattgctatcgagttcgtgctcaaccgcggacggatggtgctgttcgatagctatcaggggctggataccggcgacctgcgcgacctgcgcaccttcgacgaattcgacgcggcggtgaaacagcagatcgcccatatcgtgcgcctgtcggccatcggcaccgtcatcagccagcgcgtccaccgcgatgtggcgccgaaaccgctgatgtcgctgctggtggaaggctgcatggagagcggcaaagatgtcgccgccggcggcgcgatggtcaaccacggtccggggctgattttctccggcctggcgacctacgtcgactcgatggcggcgatccgcaagctggtgttcgaagagaagaaatacacccttgagcagatccgcgatgcgctgctggccaactttgaaggttacgaagcgctgcgccgcgactgcctgaacgcgccgaaatacggtaacgacgataactacgtcgaccagtacgcgctggatattaccgaatggaccgagaaagagtgccgtaagtacaaaatgctctactcgaccctcagccacggcaccctgtctatctccaacaacacgccaatcggcgagctgaccaacgccacgccgaacggccgcctggcgtggatgccgctctccgacggcatcagcccgactcagggcgcggataaacaaggcccgacggcgattatcaagtcggtcagcaagatgaacgtggagaccatgaacatcggtatggtgcacaacttcaaattcctcaaagggctgctggataccccggaggggcgccatggactgattaccttgctgcgtaccgcctcgattctcggcaacggccagatgcagttcagctatgtcgataacgaagtgctgaagaaggcgcagcaggagccggagaaataccgcgacctgatcgtccgcgtcgccggctacagcgcttacttcgtcgagctgtgcaaagaggtccaggacgagatcatcagccgtacggtg

SEQ ID NO: 37 - DNA, 1148 bp, Olsenella porci
  source 1..1148: mol_type = genomic DNA
  primer_bind 7..26
  primer_bind 69..88
  primer_bind 131..148
  primer_bind 598..624
  primer_bind 787..805
  primer_bind 1122..1142
cgtgccactttgacgacacgcacatcaagatgatgctcgccaagggcgtgagcgtcgaggatgcccgcgactactgcatgatgggctgcgtcgagccccagaagtctggtcgcctgtatcagtggacctccacctcatacacccagtggcccatctgcatcgagctcaccctcaaccacggcatccccctgtggtacggcaagcaggtcacgcctgactacggtgaccctgcgcagtacaagacctacgaggagtttgacgccgcggtcaagaagaccatctactacgtgaccaagtggactgatgtcgcaaccgtgatctcgcagcgcgttgcccgcgacgtcgcccccaagcctctcatgtccatcatgtacgaggggtgcatggagcacggcaaggacgtctcggccggtggcgctatgtacaactacggccccggcgtcgtgtggacgggccttgcgacctacgccgactccatggccgccatcaagaagctcgtcttcgacgagcacaagtacaccctcacccagcttgccgagggtctcaaggccgacttcgagggctacgagcagatgcagcaggactgcctcaacgcccccaagtatggcaacgacgatgactacgccgacagcatcgcggcagacatcatcgactacaccgagcacatccacctggacttcaagacgctgtactcgcacatgtccaccggtacgctctccatctccaacaacacgcccttcggcgagatgacgggcgccacggcgaacggccgcaaggcctggacgccgctgtccgacggcatcagccccacccagggcgccgaccacaggggacccactgccatcatcaagtccgtctccaagctgtcgaacgattccatgaacatcggcatggttcataacttcaagctcatgagcggcctgctcgacacccccgagggcgagaacggcctcatcacgctgctgcgcaccgcctcgatgttcggcaatggcgagatgcagttcaactacctggacaacaagacgctcatcgatgcccagaagcaccccgagaagcaccgcgacctggtcgtgcgcgtcgccggctactccgcgttcttcaacgagctctgcaaggacgtccaggacgagatcatcagccgcaccatg

SEQ ID NO: 38 - DNA, 1148 bp
cctgccacttcgacgacgcccacatcaagatgatgctggcaaagggcgtgagcatcgaggatgccagagactactgtctgatgggctgcgtggagccgcagaaatcgggccgtctctatcagtggacctccaccgcatatacccagtggccggtctgcatcgaactggtgttaaaccatggcgttccgctctggtacggcaaacaggtctgcccggacatgggagatttgagccggtttaagacctttgaggaatttgacgcagccgtaaaggaagagattaaatacgtgacaaaatggaccgacgtggctacggtgatttcccagagagtccataaggaactggctccgaagccgctgatgtcgatcatgtacgagggctgtatggagaaaggaaaagacgtttcctccggcggtgcgatgtataattacggcccgggtgtcgtatggtcgggtctcgccacctacaccgactccatggccgccatcaaaaagctggtatttgatgataagaagtacacactggagcagctaaacgaagcgttaaaagcggatttcgttggatacgaccagatcaaagcagactgcttaaacgctccgaagtacggcaacgatgatgattacgcagatctcatcgcagcggatttagttgattttacggaggcggagcacagaaaatacaagacgctgtattcccatttaagccacggcacgctgtccatctctaacaatacaccgtttgggcagatgacaggggcttcggccaacggccggggcgcatggctcccgttatccgacggcatcagcccaacccagggtgcggactacaaggggccgacggctatcattaagtcggtgtccaagatggcaaacgacagcatgaacatcggtctggtacataactttaagatcatggcaggcctcttagacactccggaaggggaagagagcctgatcaccctgctccgtaccgccagcattttcggaaacggcgagatgcagtttaactatctggataacaatacgctcctggaagctcagaagcatccggagaaataccgtgacttaatcgtccgggtagccggatacagcgcctttttcgtggaactctgcaaggaggttcaggatgagattatcagcagaaccatg

SEQ ID NO: 39 - DNA, 1156 bp, Proteus mirabilis
  source 1..1156: mol_type = genomic DNA
  primer_bind 7..26
  primer_bind 69..87
  primer_bind 131..148
  primer_bind 598..624
  primer_bind 787..805
  primer_bind 1122..1142
cctgtcacttcgatgattctcatatcaagatgatgttgcgcaaaggcttcgactttgaagatgcacgcgattactgcttgatgggctgtgttgaaccacaaaaatcaggtcgtatctatcaatggacatcaacgggttatacccagtggccaattgccattgaatttgtattaaatcgtggtcgtatggtgctgtttgatagctaccaaggcttagacaccggcgatttacgtgatttacgtacttatgaggatttcgatcgcgcggttaaagagcaagtcgcacatattattcgtttatcagcaattggtacggttatcagccagcgcgttcaccgtgacattgccccaaaaccactcatgtcgctattggttgaaggttgtatggagcaaggtaaagacgtgacagcgggtggtgcgatggttaaccacggaccgggtctgatcttctctggtttagccacttatgtcgattctatggcggcaattcgcaaactggtttatgaagacaaaaaatataccttagagcaaatacgtgacggcttattagctaattttgaagggcacgaagagttactgcgtgactgtttaaatgcaccgaaatttggtaacgacgatgatgttgttgaccaatatgcgttagacattaccgaatggactgaacgtgaatgccgtaaatataaaatgctctactccacatttagtcacggtacgttatctatctctaataacacgccaattggtgaattaaccgcagcaacaccaaacggtcgtttagcatggaaaccattatcagatgggatcagccctacacagggtgccgataaacatggcccaactgccatcattaaatccatcagcaagatgaatgttgaaaccatgaatatcggtatggttcataactttaaattcctcaaaggcttgctagataccaatgaaggacgccaaggattaattaccttattaagaactgcctctattttgggtaatggtcagatgcaatttagctatgtcgataatgaagtactgaaaaaagcccaattagagcctgaaaagtaccgcgatttaattgtccgggttgctggctacagtgcgtacttcgttgaattatgtaaagaagttcaggatgaaattattagtcgtacagtgattgagaa

SEQ ID NO: 40 - DNA, 20 bp, synthetic construct
  source 1..20: mol_type = other DNA; note = Primer
acttygaygaydcbcacatc

SEQ ID NO: 41 - DNA, 20 bp, synthetic construct
  source 1..20: mol_type = other DNA; note = Primer
gaytactgyhtsatgggytg

SEQ ID NO: 42 - DNA, 18 bp, synthetic construct
  source 1..18: mol_type = other DNA; note = Primer
cacsksmtayacccagtg

SEQ ID NO: 43 - DNA, 18 bp, synthetic construct
  source 1..18: mol_type = other DNA; note = Primer
csaartwyggyaacgayg

SEQ ID NO: 44 - DNA, 22 bp, synthetic construct
  source 1..22: mol_type = other DNA; note = Primer
tayggyaacgaygatraytayg

SEQ ID NO: 45 - DNA, 19 bp, synthetic construct
  source 1..19: mol_type = other DNA; note = Primer
cgytntccgacggyatcag

SEQ ID NO: 46 - DNA, 21 bp, synthetic construct
  source 1..21: mol_type = other DNA; note = Primer
caggaygaratyatyagymgh

SEQ ID NO: 47 - DNA, 20 bp, synthetic construct
  source 1..20: mol_type = other DNA; note = Primer
carcccatsadrcagtartc

SEQ ID NO: 48 - DNA, 18 bp, synthetic construct
  source 1..18: mol_type = other DNA; note = Primer
crtcgttrccrwayttsg

SEQ ID NO: 49 - DNA, 22 bp, synthetic construct
  source 1..22: mol_type = other DNA; note = Primer
crtartyatcrtcgttrccrta

SEQ ID NO: 50 - DNA, 19 bp, synthetic construct
  source 1..19: mol_type = other DNA; note = Primer
ctgatrccgtcgganarcg

SEQ ID NO: 51 - DNA, 1300 bp, Clostridium saccharolyticum
  source 1..1300: mol_type = genomic DNA
  primer_bind 7..32
  primer_bind 476..502
  primer_bind 1215..1235
  primer_bind 1266..1285
gaaaatcggttgatgaatattgtgaggaccagtaccgggaagccggggtatgggaattatccggggaatcctttgtatctgactgctcctaccatgccatcaacggcggcggtgactccaacccgggctatgatgtgattcttatgaagaagggcatgctggacattcagcaggaagccaaggatcatttaaaagaactggattatgagaatccggatgatattgaaaagatttatttttacaaatccattatcgataccacagaaggcgttatgatctatgcaaaaaggctttctgagtatgcagcggagcttgcggcaaaggaaaccaatccaaagcgtaaggaagagctgttaaagatctcagaagtaaatgcttacgttcctgctcacaagcccagaaccttctgggaagcgatccaggccgtatggaccattgaatccctccttgtagtggaagagaaccagaccggtatgtccatcggacgtgtggatcagtatatgtatccattctacaaagacgatatcgaatccggccggatgaatgattaccaggcatttgagcttgccggctgcatgctgatcaaaatgtctgagatgatgtggatcaccagcgaaggcggttccaaattctttgcaggctaccagccgttcgtaaacatgtgcgtaggcggtgtgacccgcagcggacatgatgccaccaatgatttaacttacttgcttatggatgccgtccgtcatgtaaagatttaccagccgtctcttgcatgccgtatccacaacaagtccccgaaaaagtacatgaaaaagatcgtggatgtggttcgttccggtatgggattcccggcttgccattttgacgacgcccacatcaagatgatgcttgcaaaaggcgtatccattgaagatgcacgtgattactgcctcatgggctgcgtagagcctcagaagtccggccgactgtatcagtggacctccactgcttatacccagtggcccatctgcatcgagcttgttttaaaccacggcgctcctttatggtatggcaagcaggtttgcccggatatgggtgacttaagcaatttcaaaacttatgaagagtttgaagctgccgtaaaagaagagatcaaatacattacaaagtggaccgatgttgccaccgtaatttcccagcgggttcacagagacttagctccaaagccgctcatgtccattatgtacgaaggctgtatggaaaaggcaaaggatgtatctgcaggcggcgccatgtacaacttcggacctggtgtggtatggtctgg

SEQ ID NO: 52 - DNA, 1291 bp, Enterocloster clostridioformis
  source 1..1291: mol_type = genomic DNA
  primer_bind 7..32
  primer_bind 476..502
  primer_bind 1215..1235
  primer_bind 1266..1285
gcaaatctgttgacgagtactgcgaggatcagtatcgcgaggctggtgtctgggagctgtccggcgagtccttcgtatcagattgttcctaccatgcaatcaacggcggtggagattccaacccgggttacgacgtgatcctgatgaagaagggcatgcttgacatccagaacgaggcgaaggagcatctggtagcacttcactatgacaatccggaggatatcgacaagatctatttctataagtcgatcatcgagacgaccgagggcgttatgatctatgcgaaaagaatgtctgagtacgcaagagagcttgctgagaaagagactgatccgaagagaaaggcagagctgtacaagatctctgaggtcaacgcaaaggttccggcacacaaaccggagacgttctgggaggcgattcaggcagtgtggacaatcgagtctctgcttgttgttgaggagaaccagaccggtatgtccatcggacgtgtcgatcagtacatgtatccgttctacaaggcagatatcgagtccggacgcatgaacaactttgaggcatttgagcttgctggatgtatgctgatcaagatgtctgagatgatgtggattacaagtgagggcggttccaagttcttcgcaggttatcagccgttcgtcaatatgtgcgtcggcggtgtgacgagagccggtcacgatgcgacaaacgacctgacctacctgctgatggatgcggttcgtcacgtaaagatttaccagccgtctctggcttgccgtattcacaacaagtccccgcgccgttatctgaagaagattgttgatgtcgtacgcgcaggaatgggattcccggcatgtcacttcgatgacactcacatcaagatgatgctcgcaaagggcgtttcgctcgaggatgcaagagattactgcctgatgggatgcgtagaaccgcagaagtccggtcgtctgtatcagtggacttccaccgcttacacccagtggccgatctgtatcgagcttgtgctcaaccacggtgttccgctgtggtacggcaagcaggtttgcccggatatgggagatttaagccagttcaagactttcgagcagtttgatgcagcagtcaaggaagagatcaagtacatcacaaagtggacggatgttgcaaccgtgatctcccagagagttcaccgcgatttagctccgaagcctttaatgtccgttatgtacgagggatgtatggagcacggaaaagacgtatctgcaggcggagccatgtataacttcggaccgggtgttgt

SEQ ID NO: 53 - DNA, 1291 bp, Clostridium carboxidivorans
  source 1..1291: mol_type = genomic DNA
  primer_bind 7..32
  primer_bind 476..502
  primer_bind 1215..1235
  primer_bind 1266..1285
gaaaatcagttgatgaatactgtgaagatcagtatcgtgaagctggagtatgggaactttcaggagaatcctttgtttcagattgttcataccacgcagtaaatggtggaggagactctaacccaggatatgacgttatcttaatgaaaaaaggtatgcttgacataaagagagaagcagaggataaattagctgagcttaattatgaaaatccagaagacatagacaaaatctatttttataaatcattaattgatactgctgaaggtgttatgatatatgctaaacgtatgtcagactatgcagctgaacttgctgcaaaggaaaccaaccctaagcgtaaagcagaacttcaaaagatttctgaagtaaatgctagagttccggcacataaaccaagtacttactgggaagcaattcaatcagtttggactatagaatcattacttgtagttgaagaaaatcaaacaggtatgtctataggacgtgttgaccaatacatgtatccattctataaagctgatattgaagctggacgtatgactgattttgaagcatttgaactatcaggttgtatgcttataaaaatgtctgaaatgatgtggataacaagtgaaggtggctctaaattctttgcaggttatcagccatttgttaacatgtgtttaggtggtgttactagagaaggacgtgatgctacaaacgacttaacttatcttttaatggatgcagttcgtcatgttaaaatatatcaaccatctttagcatgtcgtatacacaaagcatcaccacagaaataccttaagaaaatagtggatgttatccgtgcaggtatgggattcccagcatgtcactttgatgatgttcatataaaaataatgttagctaaaggtgtttctatagaagatgcaagagattactgcttaatgggatgcgttgaacctcagaaggcaggaagattatatcaatggacttctacaggatatactcaatggcctatatgtatagaacttgttcttaaccatggtgtaccgctatggtatggtaagcaagtgtgcccaaatttaggagacttaagcaactttaaaacttatgaacagtttgaagctgctgttaaagagcaaattaaatacatcactaaatggacaagtgttgctacagtaatttctcaacgtgttcacaaagatcttgcaccaaaaccacttatgtctatgatgtatgaaggctgtatggaaaagggtagaggagtagaagcaggcggagctatgtataacttcggacctggagtagt

SEQ ID NO: 54 - DNA, 1290 bp, Clostridium ljungdahlii
  source 1..1290: mol_type = genomic DNA
  primer_bind 7..32
  primer_bind 476..502
  primer_bind 1215..1235
  primer_bind 1266..1284
gaaaatctgttgatgaatactgtgaagaccagtaccgtgaagcaggtgtttgggaactttctggtgaatcatttgtttcagattgctcttaccatgcaactaatggtggtggagattcaaaccctggatatgatgttatcttaatgaaaaaaggtatggcagatattcagcaggaagcaaaggatcatttagcaaaattagattatgaaaatcctgaagatatcgaaaagatttatttctataaatccgttattgatactactgaaggagttatgatttacgctaaacgtatgtctgaatatgctgctgaattagctgcaaaggagacaaaccctaaacgtaaggcagaattacaaaagatttcagaagttaatgctcatgttcctgcacataagcctagcaatttctgggaagcaattcaatcagtttggactattgagtcattactcgtagttgaagaaaaccaaactggtatgtcaatcggccgtgttgaccaatatatgtatccattctataaggcagatatagaatcaggacgtatgaataattatgaagcatttgaattagctggttgtatgttaatcaaaatgtctgaaatgatgtgggttacaagcgaaggtgcttctaagttctttgcaggttaccaaccattcgtaaatatgtgtgttggtggtgttactcgtgacggtcttgatgcaacaaatgacttgacttatcttttgatggatgctgttcgtcacgttaagatttatcagccatctttagcttgtcgtattcacaacaaatcacctaagaagtacttgaagaagattgttgatgttgttcgtgctggtatgggattcccagcttgccattttgatgatgcacatattaagatgatgcttgcaaaaggtgtttccatagaagatgctagagattattgtataatgggttgtgttgagcctcagaaagctggacgtttatatcagtggacttctacagcttatactcaatggcctatatgtatagaattagttctaaaccatggtgttcctttatggtatggaaaacaagtttgtcctgatatgggagatttaaatagatttaagacttatgaagagtttgatgctgctgttaaggaagaaatcaaatatattacaaaatggactgacgttgctacagttatttctcagcgtgttcacagagatttagctccaaaacctttgatgtccatcatgtatgaaggctgtatggaacacggtaaagatgtttctgccggtggtgctatgtacaatttcggacctggtgttg

SEQ ID NO: 55 - DNA, 26 bp, synthetic construct
  source 1..26: mol_type = other DNA; note = Primer
cdgttgaygartaytgygargaycag

SEQ ID NO: 56 - DNA, 27 bp, synthetic construct
  source 1..27: mol_type = other DNA; note = Primer
gtchatmggmcgtgtbgaycartayat

SEQ ID NO: 57 - DNA, 21 bp, synthetic construct
  source 1..21: mol_type = other DNA; note = Primer
atgtaygarggmtgtatggar

SEQ ID NO: 58 - DNA, 20 bp, synthetic construct
  source 1..20: mol_type = other DNA; note = Primer
atgtayaayttcggacckgg

SEQ ID NO: 59 - DNA, 27 bp, synthetic construct
  source 1..27: mol_type = other DNA; note = Primer
atrtaytgrtcvacacgmccmatdgac

SEQ ID NO: 60 - DNA, 21 bp, synthetic construct
  source 1..21: mol_type = other DNA; note = Primer
ytccatacakccytcrtacat

SEQ ID NO: 61 - DNA, 20 bp, synthetic construct
  source 1..20: mol_type = other DNA; note = Primer
ccmggtccgaarttrtacat

SEQ ID NO: 62 - DNA, 318 bp, Escherichia coli
  source 1..318: mol_type = genomic DNA; strain = MEI003
  primer_bind 7..29
  primer_bind 283..312
tgcccatatcatgcctgggcattcaaactcgatggcaatctggcccatgcacgtaactgcgaaaacgtcgccaatttcgatagcgacaaagcgcaactggttccggtgcgtctggaagaatatgccggattcgtcttcatcaacatggaccctaacgccaccagcgtagaagatcagttacccggtctgggggcgaaagtgctggaagcctgcccggaagtccacgacctgaaactggcggcccgctttaccacccgcacgcctgccaactggaagaacattgtcgataactatctcgagtgctatcactgtggtccg

SEQ ID NO: 63 - DNA, 317 bp, Citrobacter portucalensis
  source 1..317: mol_type = genomic DNA
  primer_bind 7..29
  primer_bind 283..311
tgcccttaccacgcatgggcgttcaaacttgacggcaatctggcgcatgcgcgtaactgcgaaaatgtcgccaacttcgacagcgaaaaagcgcaccttacacctgtacgtctggaagagtatgccggattcgtgtttatcaacatggatccgaacgcgggcagcgtggaagaacaactcccaggtcttgcagacaaagttatcgaagcctgccctgatgtgcatgacctgaagctggcggcgcgctttacgacccgaactccagccaactggaagaatattgtcgataactatctggagtgctaccactgtggccc

SEQ ID NO: 64 - DNA, 318 bp, Klebsiella pneumoniae
  source 1..318: mol_type = genomic DNA
  primer_bind 7..29
  primer_bind 283..312
tgcccctatcacgcctgggccttcaagctggacggcaatctcgcccacgcccgcaactgcgaaaacgtggcgaatttcgatagcgaaaaggcaacgctggtgccggttcgcctggaagagtatgccggctttgtgtttatcaatatgaatccggaagcggagagtgtggaaacgcagctaccggggctgcaggacaaagtgctggaagcctgtccggacgttcatgatctgaaactggcggcgcgctttaccaccctcaccccggcgaactggaaaaatatcgtcgataactatctggaatgttaccactgcggtccg

SEQ ID NO: 65 - DNA, 23 bp, synthetic construct
  modified_base 9: mod_base = i
  modified_base 15: mod_base = i
  source 1..23: mol_type = other DNA; note = Primer
taycaygcntggrcnttyaarct

SEQ ID NO: 66 - DNA, 30 bp, synthetic construct
  source 1..30: mol_type = other DNA; note = Primer
rcagtgrtarcaytcsakrtagttrtcrac

SEQ ID NO: 67 - DNA, 288 bp, Eubacterium rectale
  source 1..288: mol_type = genomic DNA
  primer_bind 9..26
  primer_bind 262..280
cgaaaaagtttttgccacatatcccaatgaatgagtatccagcaggagcattaacggctgctttatatttgtgtagcggtatacgtgcaatggagagaggtacaatttcagaaggaagaaatgaagatggtagcgacaaattggctgatatggaattagtgcgtatagcaatacctagacgagtgtattcattatctcatgttaaatatgcaattgatagattaaaatggttgtttgataatagagagttgatacagggattggaatttgttgaagaaccagaaaaat

SEQ ID NO: 68 - DNA, 284 bp, Akkermansia muciniphila
  source 1..284: mol_type = genomic DNA
  primer_bind 7..23
  primer_bind 260..278
gggcgtttcctgccccatatcccgcaggaggactatcccgccggggctttggcggcggctttcttcatcgcctccggcgtgcgcggcatggaacgcggcacgctttccagcgtccgcgacgaaaacggcaaggacattctggcggatgtggaactgctccgcctggccttcccgcgccgtgtcttcacattatcccaggtgaaatacgtggcggaccgcatgaagtggctctatgacaaccgcgatttgattggcggcctggaatttgtggaggaaccgcccgt

SEQ ID NO: 69 - DNA, 17 bp, synthetic construct
  source 1..17: mol_type = other DNA; note = Primer
ttyytgccmcatatccc

SEQ ID NO: 70 - DNA, 19 bp, unidentified
  source 1..19: mol_type = other DNA; note = Primer
ggttcytcmacaaattcca

SEQ ID NO: 71 - DNA, 350 bp, Bacteroides thetaiotaomicron
  source 1..350: mol_type = genomic DNA
atggaattaccttttgctgaatcatggaaaatcaagatggtagaacccatcagaaaaagtacccgcgaagaacgcgagcaatggattaaagaagcacattataacgtctttcaactcaaatcagagcaagtttatattgatcttatcaccgactccggaacgggagccatgagcgaccgccaatgggcaggcatgatgctgggtgatgaaagttatgccggtgccacctccttcttcaaactaaaagataccattacaagaataacaggattcgaatacatcattcctacccatcaaggacgggcagcagaaaatgttcttttctcttatctggtacatgaaggcaatat

SEQ ID NO: 72 - DNA, 350 bp, Bacteroides ovatus
  source 1..350: mol_type = genomic DNA
atggaattaccttttgctgaatcatggaaaatcaagatggtagaacccatccggaaaagcacacgtgaagagcgtgagcaatggattaaagaagcacattataatgtctttcaactcaaatcagaacaagtttatatcgatctcatcaccgactccggcaccggagcgatgagtgaccgtcaatgggcgggaatgatgctaggtgatgaaagctatgccggagcgacctcattcttcaagttgaaagagatgattacgaaactaacaggatttgaatacatcataccaacccatcagggacgtgccgctgaaaatgttcttttctcttatttggtacatgaaggagacat

SEQ ID NO: 73 - DNA, 350 bp, Bacteroides xylanisolvens
  source 1..350: mol_type = genomic DNA
atggaattaccttttgctgaatcatggaaaataaagatggtagaacccatccggaaaagcacacgtgaagaacgcgagcaatggattaaagaagcacattataatgtctttcaactcaaatcagaacaagtttatatcgatctcatcaccgattccggaaccggagcgatgagcgaccgtcaatgggcgggaatgatgctaggcgatgaaagctacgccggagcaacctctttctttaagttgaaagagatgattacgaaactgacaggatttgaatatatcatacctacccatcaaggacgtgccgcagaaaatgtgcttttctcttatctcgtgcatgaaggagacat

SEQ ID NO: 74 - DNA, 667 bp, Porphyromonas asaccharolytica
  source 1..667: mol_type = genomic DNA
ctcaaggagggcgacatcgtaccgggtaactcgcactttgacacgacaaaggggcatatcgagtttcgcaaggctgtagccgtcgactgcacgatcgatgcagcgagcaacacggagctagagctacccttcaagggtgagatggatctgaacaagctggaggattgcttcaagaagtatcccaaggagcagatccctatgtgcgtcctgacggtgaccaacaacacggctggcggtcagcctgtctctatgaagaatgtacgtgagacgagtgagctgtgccacaagtacggcataccgctacagatcgatggtgctcgctttgctgagaatgcttacttcatcaagatgcgtgaggagggctatgcggacaagtcgatcaaggagatcgtccgtgagatgctcagctacgctgacatcatgaccatgtctagcaagaaggacgctgtggtcaacatgggtggcttcctcgctatgcgtgacgaggagctctatcacaagtgctctatgtacgctgtgatgaatgagggcttcctgacctacggcggtatgaacggtcgtgatatgaacgcgctcgctattggtctggatgagaacacggagtttgacatgctcgacacgcgtatccgtcaggtggcttacctcggtagcaagctagacgagtacg

SEQ ID NO: 75 - DNA, 245 bp, Alistipes finegoldii
  source 1..245: mol_type = genomic DNA
tgctcaaagagggcgacatcgtgccgggcaattcccatttcgacaccacgaagggacacatcgagttccgccgctgccacgccgtggactgcaccatcgacgaggcggccgacacccagaaggagctgccgttcaaaggcgaaatggacatcgccaagctcgaaaagctcctgcgcgagaacccgcgcgagaaagttccgtgcgtggtgctgaccatcaccaacaacacggcgggcggacagccc

SEQ ID NO: 76 - DNA, 284 bp, Clostridium saccharolyticum
  source 1..284: mol_type = genomic DNA
  primer_bind 7..25
  primer_bind 252..278
tattccggaaccgttcagaattaaaatggtagaacgtattaaaatgttaacacaagaagaacgtattgaaaaaatcaaagaggctaagtataatttgtttaatcttaggggagaagatgtctatattgaccttctaaccgacagcggaaccaatgctatgagcgatggccaatgggcaggcgtcatgaggggagatgaagcatacgccggttcatccagttactttaaattaattgatgcaggtaaagatatattcggttatgattatatacagccggttcatc

SEQ ID NO: 77 - DNA, 350 bp, Clostridium sordellii
  source 1..350: mol_type = genomic DNA
  primer_bind 21..39
  primer_bind 269..292
atgagtaaaaaatacgtagcagaaccattcaaaatcaaaatggtagaaccaatcaaaatgacaacaaaagaggaaagagaagtaaagatagcaaatgcaaattataacttattttcattaaaagcagatgatgtgtacatagacttattaactgatagtgggactggtgctatgagttcaaagcaatgggcagcagttatgttaggagacgagtcatattcaggggctagtagctactttaaattagtagatgcagctaaagatatttttggatataaatatatacaaccagtacatcaaggtagagcggctgaaaaggttttaattcctttgtttgctgagactgggaa

SEQ ID NO: 78 - DNA, 19 bp, synthetic construct
  source 1..19: mol_type = other DNA; note = Primer
rgaaccrttcaraatyaaa

SEQ ID NO: 79 - DNA, 24 bp, synthetic construct
  source 1..24: mol_type = other DNA; note = Primer
cyggytgtatatawryatawccra

SEQ ID NO: 80 - DNA, 21 bp, synthetic construct
  source 1..21: mol_type = other DNA; note = Primer
gctcaagatttccgaggtcaa

SEQ ID NO: 81 - DNA, 19 bp, synthetic construct
  source 1..19: mol_type = other DNA; note = Primer
gcaccagttcgatgcagat

SEQ ID NO: 82 - DNA, 22 bp, synthetic construct
  source 1..22: mol_type = other DNA; note = Primer
caatctgagccctgactttgta

SEQ ID NO: 83 - DNA, 21 bp, synthetic construct
  source 1..21: mol_type = other DNA; note = Primer
acatcgcgataccactcaatc

SEQ ID NO: 84 - DNA, 20 bp, unidentified
  source 1..20: mol_type = other DNA; note = Primer
aacgtaccactcgcgcttat

SEQ ID NO: 85 - DNA, 20 bp, synthetic construct
  source 1..20: mol_type = other DNA; note = Primer
agttttgcggtgaagtgacg

SEQ ID NO: 86 - DNA, 16 bp, synthetic construct
  source 1..16: mol_type = other DNA; note = Primer
actgagacacggccca

SEQ ID NO: 87 - DNA, 19 bp, synthetic construct
  source 1..19: mol_type = other DNA; note = Primer
ttaccgcggcmgctggcac

SEQ ID NO: 88 - DNA, 18 bp, synthetic construct
  source 1..18: mol_type = other DNA; note = Probe
actcctacgggaggcagc

SEQ ID NO: 89 - DNA, 50 bp, synthetic construct
  source 1..50: mol_type = other DNA; note = Primer
tcgtcggcagcgtcagatgtgtataagagacagcctacgggnggcwgcag

SEQ ID NO: 90 - DNA, 55 bp, synthetic construct
  source 1..55: mol_type = other DNA; note = Primer
gtctcgtgggctcggagatgtgtataagagacaggactachvgggtatctaatcc

SEQ ID NO: 91 - DNA, 159 bp, Clostridium scindens
  source 1..159: mol_type = genomic DNA
  primer_bind 7..26
  primer_bind 134..153
aggattcagcccgcagatgttctttgacgagaccaacaccctggaaactccggacactcttacggtagagaggattcatgagatcgtagaagaattcggacgcggcgcaaggatggctgttcaggctggatttgacgcagtagaattccatgcggctca

SEQ ID NO: 92 - DNA, 20 bp, synthetic construct
  source 1..20: mol_type = other DNA; note = Primer
cagcccrcagatgttctttg

SEQ ID NO: 93 - DNA, 20 bp, synthetic construct
  source 1..20: mol_type = other DNA; note = Primer
gcatggaattchactgcrtc

SEQ ID NO: 94 - DNA, 23 bp, synthetic construct
  source 1..23: mol_type = other DNA; note = Primer
gggcatccagctgtggcatggag

SEQ ID NO: 95 - DNA, 20 bp, synthetic construct
  source 1..20: mol_type = other DNA; note = Primer
cgtgaggcagataactgtga

SEQ ID NO: 96 - DNA, 283 bp, Desulfovibrio desulfuricans
  source 1..283: mol_type = genomic DNA
  primer_bind 7..24
  primer_bind 250..276
gtctgactaacatgcacggttccaccggcgatatcgtgctgctcggtacccagactgcccagctggaagaaatcttccacgaactgacccacaacatgaatgttgacctgggtggttccggctccaacctgcgtacgcccgaatcctgccttggccagtcgcgctgcgaatatgcctgctacaacacgcaggacatgtgctacacgctgaccatggactatcaggacgaactgcaccgtcccgccttcccctacaagttcaagttcaagttcgacggttgccc

SEQ ID NO: 97 - DNA, 18 bp, synthetic construct
  source 1..18: mol_type = other DNA; note = Primer
ccaacatgcacggytcca

SEQ ID NO: 98 - DNA, 26 bp, synthetic construct
  source 1..26: mol_type = other DNA; note = Primer
cgtcgaattgaacttgaacttgtagg

SEQ ID NO: 99 - DNA, 21 bp, synthetic construct
  source 1..21: mol_type = other DNA; note = Primer
cgtggttctggtctgactaac

SEQ ID NO: 100 - DNA, 22 bp, synthetic construct
  source 1..22: mol_type = other DNA; note = Primer
gaaggacgacatcaagatcgac